European Patent Application EP 4 480 498 A1, published December 25, 2024. Title: Antibody-drug conjugate targeting c-Kit. Applicant: Novelty Nobility Inc. The sequence listing filed with the application follows.

SEQUENCE LISTING (12 sequences)

SEQ ID NO: 1 - protein, 8 aa, Artificial Sequence
  H-CDR1
GFTFSRYG

SEQ ID NO: 2 - protein, 8 aa, Artificial Sequence
  H-CDR2
IWYDGTNK

SEQ ID NO: 3 - protein, 11 aa, Artificial Sequence
  H-CDR3
AREDWAEAFDM

SEQ ID NO: 4 - protein, 11 aa, Artificial Sequence
  L-CDR1
QSLLHSNGYNY

SEQ ID NO: 5 - protein, 3 aa, Artificial Sequence
  L-CDR2
LGS

SEQ ID NO: 6 - protein, 8 aa, Artificial Sequence
  L-CDR3
MQALQTIT

SEQ ID NO: 7 - protein, 118 aa, Artificial Sequence
  Heavy chain variable region
QVQLVESGGGVVQPGRSLRLSCAASGFTFSRYGMHWVRQAPGKGLEWVAVIWYDGTNKDYTDSVRGRFTISRDNSKNTLYLQMNSLRAEDTAVYYCAREDWAEAFDMWGQGTTVTVSS

SEQ ID NO: 8 - protein, 111 aa, Artificial Sequence
  Light chain variable region
DIVMTQSPLSLPVTPGEPASISCRSSQSLLHSNGYNYLDWYLQKPGQSPQLLIYLGSNRASGVPDRFSGSGSGTDFTLKISRVEAEDVGVYYCMQALQTITFGQGTRLEIK

SEQ ID NO: 9 - protein, 84 aa, Artificial Sequence
  R122 to R205 in c-Kit domain 2
RSLYGKEDNDTLVRCPLTDPEVTNYSLKGCQGKPLPKDLRFIPDPKAGIMIKSVKRAYHRLCLHCSVDQEGKSVLSEKFILKVR

SEQ ID NO: 10 - protein, 24 aa, Artificial Sequence
  S240 to H263 in c-Kit domain 3
SSVYSTWKRENSQTKLQEKYNSWH

SEQ ID NO: 11 - protein, 197 aa, Artificial Sequence
  c-Kit domain 2-3 (D113 to D309)
DPAKLFLVDRSLYGKEDNDTLVRCPLTDPEVTNYSLKGCQGKPLPKDLRFIPDPKAGIMIKSVKRAYHRLCLHCSVDQEGKSVLSEKFILKVRPAFKAVPVVSVSKASYLLREGEEFTVTCTIKDVSSSVYSTWKRENSQTKLQEKYNSWHHGDFNYERQATLTISSARVNDSGVFMCYANNTFGSANVTTTLEVVD

SEQ ID NO: 12 - protein, 284 aa, Artificial Sequence
  c-Kit domain 1-3 (Q26 to D309)
QPSVSPGEPSPPSIHPGKSDLIVRVGDEIRLLCTDPGFVKWTFEILDETNENKQNEWITEKAEATNTGKYTCTNKHGLSNSIYVFVRDPAKLFLVDRSLYGKEDNDTLVRCPLTDPEVTNYSLKGCQGKPLPKDLRFIPDPKAGIMIKSVKRAYHRLCLHCSVDQEGKSVLSEKFILKVRPAFKAVPVVSVSKASYLLREGEEFTVTCTIKDVSSSVYSTWKRENSQTKLQEKYNSWHHGDFNYERQATLTISSARVNDSGVFMCYANNTFGSANVTTTLEVVD